European Patent Application EP 4 230 225 A1, published August 23, 2023. Title: ANTIBODY-DRUG CONJUGATE AND APPLICATION THEREOF. Applicant: SHANGHAI MIRACOGEN INC. KEYMED BIOSCIENCES CO.,LTD. The sequence listing filed with the application follows.

SEQUENCE LISTING (200 sequences)

SEQ ID NO: 1 - protein, 118 aa, Artificial
  18D10VHv1
QVQLQESGPGLVKPSETLSLTCTVSGYSITSNYAWNWIRQPPGKGLEWIGYINYSGNTNYNPSLKSRVTISRDTSKNQFSLKLSSVTAADTAVYYCATSYYGNSFIYWGQGTLVTVSS

SEQ ID NO: 2 - protein, 11 aa, Artificial
  18D10VHv1 CDR1
GYSITSNYAWN

SEQ ID NO: 3 - protein, 16 aa, Artificial
  18D10VHv1 CDR2
YINYSGNTNYNPSLKS

SEQ ID NO: 4 - protein, 9 aa, Artificial
  18D10VHv1 CDR3
SYYGNSFIY

SEQ ID NO: 5 - protein, 25 aa, Artificial
  18D10VHv1 FR1
QVQLQESGPGLVKPSETLSLTCTVS

SEQ ID NO: 6 - protein, 14 aa, Artificial
  18D10VHv1 FR2
WIRQPPGKGLEWIG

SEQ ID NO: 7 - protein, 32 aa, Artificial
  18D10VHv1 FR3
RVTISRDTSKNQFSLKLSSVTAADTAVYYCAT

SEQ ID NO: 8 - protein, 11 aa, Artificial
  18D10VHv1 FR4
WGQGTLVTVSS

SEQ ID NO: 9 - protein, 118 aa, Artificial
  18D10VHv2
QVQLQESGPGLVKPSETLSLTCTVSGGSISSNYAWNWIRQPPGKGLEWMGYINYSGNTNYNPSLKSRITISRDTSKNQFSLKLSSVTAADTAVYYCATSYYGNSFIYWGQGTLVTVSS

SEQ ID NO: 10 - protein, 11 aa, Artificial
  18D10VHv2 CDR1
GGSISSNYAWN

SEQ ID NO: 11 - protein, 16 aa, Artificial
  18D10VHv2 CDR2
YINYSGNTNYNPSLKS

SEQ ID NO: 12 - protein, 9 aa, Artificial
  18D10VHv2 CDR3
SYYGNSFIY

SEQ ID NO: 13 - protein, 25 aa, Artificial
  18D10VHv2 FR1
QVQLQESGPGLVKPSETLSLTCTVS

SEQ ID NO: 14 - protein, 14 aa, Artificial
  18D10VHv2 FR2
WIRQPPGKGLEWMG

SEQ ID NO: 15 - protein, 32 aa, Artificial
  18D10VHv2 FR3
RITISRDTSKNQFSLKLSSVTAADTAVYYCAT

SEQ ID NO: 16 - protein, 11 aa, Artificial
  18D10VHv2 FR4
WGQGTLVTVSS

SEQ ID NO: 17 - protein, 118 aa, Artificial
  18D10VHv3
QVQLQESGPGLVKPSETLSLTCTVSGGSISSNYAWNWIRQPPGKGLEWIGYINYSGNTNYNPSLKSRVTISRDTSKNQFSLKLSSVTAADTAVYYCATSYYGNSFIYWGQGTLVTVSS

SEQ ID NO: 18 - protein, 11 aa, Artificial
  18D10VHv3 CDR1
GGSISSNYAWN

SEQ ID NO: 19 - protein, 16 aa, Artificial
  18D10VHv3 CDR2
YINYSGNTNYNPSLKS

SEQ ID NO: 20 - protein, 9 aa, Artificial
  18D10VHv3 CDR3
SYYGNSFIY

SEQ ID NO: 21 - protein, 25 aa, Artificial
  18D10VHv3 FR1
QVQLQESGPGLVKPSETLSLTCTVS

SEQ ID NO: 22 - protein, 14 aa, Artificial
  18D10VHv3 FR2
WIRQPPGKGLEWIG

SEQ ID NO: 23 - protein, 32 aa, Artificial; identical to SEQ ID NO: 7
  18D10VHv3 FR3

SEQ ID NO: 24 - protein, 11 aa, Artificial
  18D10VHv3 FR4
WGQGTLVTVSS

SEQ ID NO: 25 - protein, 118 aa, Artificial
  18D10VHv4
QVQLQESGPGLVKPSETLSLTCTVSGGSISSNYAWNWIRQPPGKGLEWIGYINYSGYTNYNPSLKSRVTISRDTSKNQFSLKLSSVTAADTAVYYCATSYYGNSFIYWGQGTLVTVSS

SEQ ID NO: 26 - protein, 11 aa, Artificial
  18D10VHv4 CDR1
GGSISSNYAWN

SEQ ID NO: 27 - protein, 16 aa, Artificial
  18D10VHv4 CDR2
YINYSGYTNYNPSLKS

SEQ ID NO: 28 - protein, 9 aa, Artificial
  18D10VHv4 CDR3
SYYGNSFIY

SEQ ID NO: 29 - protein, 25 aa, Artificial
  18D10VHv4 FR1
QVQLQESGPGLVKPSETLSLTCTVS

SEQ ID NO: 30 - protein, 14 aa, Artificial
  18D10VHv4 FR2
WIRQPPGKGLEWIG

SEQ ID NO: 31 - protein, 32 aa, Artificial; identical to SEQ ID NO: 7
  18D10VHv4 FR3

SEQ ID NO: 32 - protein, 11 aa, Artificial
  18D10VHv4 FR4
WGQGTLVTVSS

SEQ ID NO: 33 - protein, 118 aa, Artificial
  18D10VHv5
QVQLQESGPGLVKPSETLSLTCTVSGGSISSNYAWNWIRQPPGKGLEWIGYINYSGNTAYNPSLKSRVTISRDTSKNQFSLKLSSVTAADTAVYYCATSYYGNSFIYWGQGTLVTVSS

SEQ ID NO: 34 - protein, 11 aa, Artificial
  18D10VHv5 CDR1
GGSISSNYAWN

SEQ ID NO: 35 - protein, 16 aa, Artificial
  18D10VHv5 CDR2
YINYSGNTAYNPSLKS

SEQ ID NO: 36 - protein, 9 aa, Artificial
  18D10VHv5 CDR3
SYYGNSFIY

SEQ ID NO: 37 - protein, 25 aa, Artificial
  18D10VHv5 FR1
QVQLQESGPGLVKPSETLSLTCTVS

SEQ ID NO: 38 - protein, 14 aa, Artificial
  18D10VHv5 FR2
WIRQPPGKGLEWIG

SEQ ID NO: 39 - protein, 32 aa, Artificial; identical to SEQ ID NO: 7
  18D10VHv5 FR3

SEQ ID NO: 40 - protein, 11 aa, Artificial
  18D10VHv5 FR4
WGQGTLVTVSS

SEQ ID NO: 41 - protein, 118 aa, Artificial
  18D10VHv6
QVQLQESGPGLVKPSETLSLTCTVSGGSISSNYAWNWIRQPPGKGLEWIGYIYYSGNTNYNPSLKSRVTISRDTSKNQFSLKLSSVTAADTAVYYCATSYYGNSFIYWGQGTLVTVSS

SEQ ID NO: 42 - protein, 11 aa, Artificial
  18D10VHv6 CDR1
GGSISSNYAWN

SEQ ID NO: 43 - protein, 16 aa, Artificial
  18D10VHv6 CDR2
YIYYSGNTNYNPSLKS

SEQ ID NO: 44 - protein, 9 aa, Artificial
  18D10VHv6 CDR3
SYYGNSFIY

SEQ ID NO: 45 - protein, 25 aa, Artificial
  18D10VHv6 FR1
QVQLQESGPGLVKPSETLSLTCTVS

SEQ ID NO: 46 - protein, 14 aa, Artificial
  18D10VHv6 FR2
WIRQPPGKGLEWIG

SEQ ID NO: 47 - protein, 32 aa, Artificial; identical to SEQ ID NO: 7
  18D10VHv6 FR3

SEQ ID NO: 48 - protein, 11 aa, Artificial
  18D10VHv6 FR4
WGQGTLVTVSS

SEQ ID NO: 49 - protein, 113 aa, Artificial
  18D10VLv1
DIVMTQSPDSLAVSLGERATINCKSSQSLLNSGNQKNYLTWYQQKPGQPPKLLIYWASTRESGVPDRFSGSGSGTDFTLTISSLQAEDVAVYYCQNAYSFPWTFGQGTKVEIK

SEQ ID NO: 50 - protein, 17 aa, Artificial
  18D10VLv1 CDR1
KSSQSLLNSGNQKNYLT

SEQ ID NO: 51 - protein, 7 aa, Artificial
  18D10VLv1 CDR2
WASTRES

SEQ ID NO: 52 - protein, 9 aa, Artificial
  18D10VLv1 CDR3
QNAYSFPWT

SEQ ID NO: 53 - protein, 23 aa, Artificial
  18D10VLv1 FR1
DIVMTQSPDSLAVSLGERATINC

SEQ ID NO: 54 - protein, 15 aa, Artificial
  18D10VLv1 FR2
WYQQKPGQPPKLLIY

SEQ ID NO: 55 - protein, 32 aa, Artificial
  18D10VLv1 FR3
GVPDRFSGSGSGTDFTLTISSLQAEDVAVYYC

SEQ ID NO: 56 - protein, 10 aa, Artificial
  18D10VLv1 FR4
FGQGTKVEIK

SEQ ID NO: 57 - protein, 113 aa, Artificial
  18D10VLv2
DIVMTQSPDSLAVSLGERATINCKSSQSLLNSGNQKNYLAWYQQKPGQPPKLLIYWASTRESGVPDRFSGSGSGTDFTLTISSLQAEDVAVYYCQQAYSFPWTFGQGTKVEIK

SEQ ID NO: 58 - protein, 17 aa, Artificial
  18D10VLv2 CDR1
KSSQSLLNSGNQKNYLA

SEQ ID NO: 59 - protein, 7 aa, Artificial
  18D10VLv2 CDR2
WASTRES

SEQ ID NO: 60 - protein, 9 aa, Artificial
  18D10VLv2 CDR3
QQAYSFPWT

SEQ ID NO: 61 - protein, 23 aa, Artificial
  18D10VLv2 FR1
DIVMTQSPDSLAVSLGERATINC

SEQ ID NO: 62 - protein, 15 aa, Artificial
  18D10VLv2 FR2
WYQQKPGQPPKLLIY

SEQ ID NO: 63 - protein, 32 aa, Artificial; identical to SEQ ID NO: 55
  18D10VLv2 FR3

SEQ ID NO: 64 - protein, 10 aa, Artificial
  18D10VLv2 FR4
FGQGTKVEIK

SEQ ID NO: 65 - protein, 448 aa, Artificial
  Heavy Chain Amino Acid Sequence
QVQLQESGPGLVKPSETLSLTCTVSGGSISSNYAWNWIRQPPGKGLEWIGYIYYSGNTNYNPSLKSRVTISRDTSKNQFSLKLSSVTAADTAVYYCATSYYGNSFIYWGQGTLVTVSSASTKGPSVFPLAPSSKSTSGGTAALGCLVKDYFPEPVTVSWNSGALTSGVHTFPAVLQSSGLYSLSSVVTVPSSSLGTQTYICNVNHKPSNTKVDKRVEPKSCDKTHTCPPCPAPELLGGPSVFLFPPKPKDTLMISRTPEVTCVVVDVSHEDPEVKFNWYVDGVEVHNAKTKPREEQYNSTYRVVSVLTVLHQDWLNGKEYKCKVSNKALPAPIEKTISKAKGQPREPQVYTLPPSREEMTKNQVSLTCLVKGFYPSDIAVEWESNGQPENNYKTTPPVLDSDGSFFLYSKLTVDKSRWQQGNVFSCSVMHEALHNHYTQKSLSLSPGK

SEQ ID NO: 66 - protein, 220 aa, Artificial
  Light Chain Amino Acid Sequence
DIVMTQSPDSLAVSLGERATINCKSSQSLLNSGNQKNYLTWYQQKPGQPPKLLIYWASTRESGVPDRFSGSGSGTDFTLTISSLQAEDVAVYYCQNAYSFPWTFGQGTKVEIKRTVAAPSVFIFPPSDEQLKSGTASVVCLLNNFYPREAKVQWKVDNALQSGNSQESVTEQDSKDSTYSLSSTLTLSKADYEKHKVYACEVTHQGLSSPVTKSFNRGEC

SEQ ID NO: 67 - protein, 118 aa, Artificial
  18A9VHv1
QVQLVQSGAEVKKPGSSVKVSCKPSGYAFTNYLIDWVRQAPGQGLEWMGGINPGSGDTVYNEKFQGRVTLTADKSSMTAYMELSSLRSEDTAVYFCARRVRGNSFDSWGQGTLVTVSS

SEQ ID NO: 68 - protein, 10 aa, Artificial
  18A9VHv1 CDR1
GYAFTNYLID

SEQ ID NO: 69 - protein, 16 aa, Artificial
  18A9VHv1 CDR2
GINPGSGDTVYNEKFQ

SEQ ID NO: 70 - protein, 9 aa, Artificial
  18A9VHv1 CDR3
RVRGNSFDS

SEQ ID NO: 71 - protein, 25 aa, Artificial
  18A9VHv1 FR1
QVQLVQSGAEVKKPGSSVKVSCKPS

SEQ ID NO: 72 - protein, 14 aa, Artificial
  18A9VHv1 FR2
WVRQAPGQGLEWMG

SEQ ID NO: 73 - protein, 33 aa, Artificial
  18A9VHv1 FR3
GRVTLTADKSSMTAYMELSSLRSEDTAVYFCAR

SEQ ID NO: 74 - protein, 11 aa, Artificial
  18A9VHv1 FR4
WGQGTLVTVSS

SEQ ID NO: 75 - protein, 118 aa, Artificial
  18A9VHv2
QVQLVQSGAEVKKPGSSVKVSCKPSGYTFTNYLIDWVRQAPGQGLEWMGGINPGSGDTVYNEKFQGRVTLTADESTSTAYMELSSLRSEDTAVYFCARRVRGNSFDSWGQGTLVTVSS

SEQ ID NO: 76 - protein, 10 aa, Artificial
  18A9VHv2 CDR1
GYTFTNYLID

SEQ ID NO: 77 - protein, 16 aa, Artificial
  18A9VHv2 CDR2
GINPGSGDTVYNEKFQ

SEQ ID NO: 78 - protein, 9 aa, Artificial
  18A9VHv2 CDR3
RVRGNSFDS

SEQ ID NO: 79 - protein, 25 aa, Artificial
  18A9VHv2 FR1
QVQLVQSGAEVKKPGSSVKVSCKPS

SEQ ID NO: 80 - protein, 14 aa, Artificial
  18A9VHv2 FR2
WVRQAPGQGLEWMG

SEQ ID NO: 81 - protein, 33 aa, Artificial
  18A9VHv2 FR3
GRVTLTADESTSTAYMELSSLRSEDTAVYFCAR

SEQ ID NO: 82 - protein, 11 aa, Artificial
  18A9VHv2 FR4
WGQGTLVTVSS

SEQ ID NO: 83 - protein, 118 aa, Artificial
  18A9VHv3
QVQLVQSGAEVKKPGSSVKVSCKPSGYTFTNYLIDWVRQAPGQGLEWMGGINPGSGDTVYNEKFQGRVTLTADKSSMTAYMELSSLRSEDTAVYYCARRVRGNSFDSWGQGTLVTVSS

SEQ ID NO: 84 - protein, 10 aa, Artificial
  18A9VHv3 CDR1
GYTFTNYLID

SEQ ID NO: 85 - protein, 16 aa, Artificial
  18A9VHv3 CDR2
GINPGSGDTVYNEKFQ

SEQ ID NO: 86 - protein, 9 aa, Artificial
  18A9VHv3 CDR3
RVRGNSFDS

SEQ ID NO: 87 - protein, 25 aa, Artificial
  18A9VHv3 FR1
QVQLVQSGAEVKKPGSSVKVSCKPS

SEQ ID NO: 88 - protein, 14 aa, Artificial
  18A9VHv3 FR2
WVRQAPGQGLEWMG

SEQ ID NO: 89 - protein, 33 aa, Artificial
  18A9VHv3 FR3
GRVTLTADKSSMTAYMELSSLRSEDTAVYYCAR

SEQ ID NO: 90 - protein, 11 aa, Artificial
  18A9VHv3 FR4
WGQGTLVTVSS

SEQ ID NO: 91 - protein, 118 aa, Artificial
  18A9VHv4
QVQLVQSGAEVKKPGSSVKVSCKASGYTFTNYLIDWVRQAPGQGLEWMGGINPGSGDTVYNEKFQGRVTLTADKSSMTAYMELSSLRSEDTAVYFCARRVRGNSFDSWGQGTLVTVSS

SEQ ID NO: 92 - protein, 10 aa, Artificial
  18A9VHv4 CDR1
GYTFTNYLID

SEQ ID NO: 93 - protein, 16 aa, Artificial
  18A9VHv4 CDR2
GINPGSGDTVYNEKFQ

SEQ ID NO: 94 - protein, 9 aa, Artificial
  18A9VHv4 CDR3
RVRGNSFDS

SEQ ID NO: 95 - protein, 25 aa, Artificial [sequence omitted]

SEQ ID NO: 96 - protein, 14 aa, Artificial
  18A9VHv4 FR2
WVRQAPGQGLEWMG

SEQ ID NO: 97 - protein, 33 aa, Artificial; identical to SEQ ID NO: 73
  18A9VHv4 FR3

SEQ ID NO: 98 - protein, 11 aa, Artificial
  18A9VHv4 FR4
WGQGTLVTVSS

SEQ ID NO: 99 - protein, 118 aa, Artificial
  18A9VHv5
QVQLVQSGAEVKKPGSSVKVSCKPSGYTFTNYLIDWVRQAPGQGLEWMGGINPGSGDTVYNEKFQGRVTITADESTSTAYMELSSLRSEDTAVYFCARRVRGNSFDSWGQGTLVTVSS

SEQ ID NO: 100 - protein, 10 aa, Artificial
  18A9VHv5 CDR1
GYTFTNYLID

SEQ ID NO: 101 - protein, 16 aa, Artificial
  18A9VHv5 CDR2
GINPGSGDTVYNEKFQ

SEQ ID NO: 102 - protein, 9 aa, Artificial
  18A9VHv5 CDR3
RVRGNSFDS

SEQ ID NO: 103 - protein, 25 aa, Artificial
  18A9VHv5 FR1
QVQLVQSGAEVKKPGSSVKVSCKPS

SEQ ID NO: 104 - protein, 14 aa, Artificial
  18A9VHv5 FR2
WVRQAPGQGLEWMG

SEQ ID NO: 105 - protein, 33 aa, Artificial
  18A9VHv5 FR3
GRVTITADESTSTAYMELSSLRSEDTAVYFCAR

SEQ ID NO: 106 - protein, 11 aa, Artificial
  18A9VHv5 FR4
WGQGTLVTVSS

SEQ ID NO: 107 - protein, 118 aa, Artificial
  18A9VHv6
QVQLVQSGAEVKKPGASVKVSCKPSGYAFTNYLIDWVRQAPGQGLEWMGGINPGSGDTVYNEKFQGRVTLTADKSSSTAYMELSSLRSEDTAVYFCARRVRGNSFDSWGQGTLVTVSS

SEQ ID NO: 108 - protein, 10 aa, Artificial
  18A9VHv6 CDR1
GYAFTNYLID

SEQ ID NO: 109 - protein, 16 aa, Artificial
  18A9VHv6 CDR2
GINPGSGDTVYNEKFQ

SEQ ID NO: 110 - protein, 9 aa, Artificial
  18A9VHv6 CDR3
RVRGNSFDS

SEQ ID NO: 111 - protein, 25 aa, Artificial
  18A9VHv6 FR1
QVQLVQSGAEVKKPGASVKVSCKPS

SEQ ID NO: 112 - protein, 14 aa, Artificial
  18A9VHv6 FR2
WVRQAPGQGLEWMG

SEQ ID NO: 113 - protein, 33 aa, Artificial
  18A9VHv6 FR3
GRVTLTADKSSSTAYMELSSLRSEDTAVYFCAR

SEQ ID NO: 114 - protein, 11 aa, Artificial
  18A9VHv6 FR4
WGQGTLVTVSS

SEQ ID NO: 115 - protein, 118 aa, Artificial
  18A9VHv7
QVQLVQSGAEVKKPGASVKVSCKPSGYTFTNYLIDWVRQAPGQGLEWMGGINPGSGDTVYNEKFQGRVTLTADTSTSTVYMELSSLRSEDTAVYFCARRVRGNSFDSWGQGTLVTVSS

SEQ ID NO: 116 - protein, 10 aa, Artificial
  18A9VHv7 CDR1
GYTFTNYLID

SEQ ID NO: 117 - protein, 16 aa, Artificial
  18A9VHv7 CDR2
GINPGSGDTVYNEKFQ

SEQ ID NO: 118 - protein, 9 aa, Artificial
  18A9VHv7 CDR3
RVRGNSFDS

SEQ ID NO: 119 - protein, 25 aa, Artificial
  18A9VHv7 FR1
QVQLVQSGAEVKKPGASVKVSCKPS

SEQ ID NO: 120 - protein, 14 aa, Artificial
  18A9VHv7 FR2
WVRQAPGQGLEWMG

SEQ ID NO: 121 - protein, 33 aa, Artificial
  18A9VHv7 FR3
GRVTLTADTSTSTVYMELSSLRSEDTAVYFCAR

SEQ ID NO: 122 - protein, 11 aa, Artificial
  18A9VHv7 FR4
WGQGTLVTVSS

SEQ ID NO: 123 - protein, 113 aa, Artificial
  18A9VLv1
DIVMTQSPDSLAVSLGERATINCKSSQSLLNSGNQKNYLTWYQQKPGQPPKLLIYWASTRESGVPDRFSGSGSGKDFTLTISSLQAEDVAVYYCQNNYFYPLTFGGGTKVEIK

SEQ ID NO: 124 - protein, 17 aa, Artificial
  18A9VLv1 CDR1
KSSQSLLNSGNQKNYLT

SEQ ID NO: 125 - protein, 7 aa, Artificial
  18A9VLv1 CDR2
WASTRES

SEQ ID NO: 126 - protein, 9 aa, Artificial
  18A9VLv1 CDR3
QNNYFYPLT

SEQ ID NO: 127 - protein, 23 aa, Artificial
  18A9VLv1 FR1
DIVMTQSPDSLAVSLGERATINC

SEQ ID NO: 128 - protein, 15 aa, Artificial
  18A9VLv1 FR2
WYQQKPGQPPKLLIY

SEQ ID NO: 129 - protein, 32 aa, Artificial
  18A9VLv1 FR3
GVPDRFSGSGSGKDFTLTISSLQAEDVAVYYC

SEQ ID NO: 130 - protein, 10 aa, Artificial
  18A9VLv1 FR4
FGGGTKVEIK

SEQ ID NO: 131 - protein, 113 aa, Artificial
  18A9VLv2
DIVMTQSPDSLAVSLGERATINCKSSQSLLNSGNQKNYLAWYQQKPGQPPKLLIYWASTRESGVPDRFSGSGSGTDFTLTISSLQAEDVAVYYCQQNYFYPLTFGGGTKVEIK

SEQ ID NO: 132 - protein, 17 aa, Artificial
  18A9VLv2 CDR1
KSSQSLLNSGNQKNYLA

SEQ ID NO: 133 - protein, 7 aa, Artificial
  18A9VLv2 CDR2
WASTRES

SEQ ID NO: 134 - protein, 9 aa, Artificial
  18A9VLv2 CDR3
QQNYFYPLT

SEQ ID NO: 135 - protein, 23 aa, Artificial
  18A9VLv2 FR1
DIVMTQSPDSLAVSLGERATINC

SEQ ID NO: 136 - protein, 15 aa, Artificial
  18A9VLv2 FR2
WYQQKPGQPPKLLIY

SEQ ID NO: 137 - protein, 32 aa, Artificial; identical to SEQ ID NO: 55
  18A9VLv2 FR3

SEQ ID NO: 138 - protein, 10 aa, Artificial
  18A9VLv2 FR4
FGGGTKVEIK

SEQ ID NO: 139 - protein, 118 aa, Artificial
  Clone 18D10 Heavy Chain
DVQLQESGPGLVKPSQSLSLTCTVTGYSITSNYAWNWIRQFPGNKLEWMGYINYSGNTNYNPSLKSRISITRDTSKNQFFLQLNSVTAEDTATYYCATSYYGNSFIYWGQGTLVTVSA

SEQ ID NO: 140 - protein, 11 aa, Artificial
  Clone 18D10 Heavy Chain CDR1
GYSITSNYAWN

SEQ ID NO: 141 - protein, 16 aa, Artificial
  Clone 18D10 Heavy Chain CDR2
YINYSGNTNYNPSLKS

SEQ ID NO: 142 - protein, 9 aa, Artificial
  Clone 18D10 Heavy Chain CDR3
SYYGNSFIY

SEQ ID NO: 143 - protein, 25 aa, Artificial
  Clone 18D10 Heavy Chain FR1
DVQLQESGPGLVKPSQSLSLTCTVT

SEQ ID NO: 144 - protein, 14 aa, Artificial
  Clone 18D10 Heavy Chain FR2
WIRQFPGNKLEWMG

SEQ ID NO: 145 - protein, 32 aa, Artificial
  Clone 18D10 Heavy Chain FR3
RISITRDTSKNQFFLQLNSVTAEDTATYYCAT

SEQ ID NO: 146 - protein, 11 aa, Artificial
  Clone 18D10 Heavy Chain FR4
WGQGTLVTVSA

SEQ ID NO: 147 - protein, 113 aa, Artificial
  Clone 18D10 Light chain
DIVMTQSPSSLTVTAGEKVTMSCKSSQSLLNSGNQKNYLTWYQQKPGQPPKLLIYWASTRESGVPDRFTGSGSGTDFTLTISSVQAEDLAVYYCQNAYSFPWTFGGGTKLEIK

SEQ ID NO: 148 - protein, 17 aa, Artificial
  Clone 18D10 Light chain CDR1
KSSQSLLNSGNQKNYLT

SEQ ID NO: 149 - protein, 7 aa, Artificial
  Clone 18D10 Light chain CDR2
WASTRES

SEQ ID NO: 150 - protein, 9 aa, Artificial
  Clone 18D10 Light chain CDR3
QNAYSFPWT

SEQ ID NO: 151 - protein, 23 aa, Artificial
  Clone 18D10 Light chain FR1
DIVMTQSPSSLTVTAGEKVTMSC

SEQ ID NO: 152 - protein, 15 aa, Artificial
  Clone 18D10 Light chain FR2
WYQQKPGQPPKLLIY

SEQ ID NO: 153 - protein, 32 aa, Artificial
  Clone 18D10 Light chain FR3
GVPDRFTGSGSGTDFTLTISSVQAEDLAVYYC

SEQ ID NO: 154 - protein, 10 aa, Artificial
  Clone 18D10 Light chain FR4
FGGGTKLEIK

SEQ ID NO: 155 - protein, 118 aa, Artificial
  Clone 18A9 Heavy Chain
QVQLQQSGREVVRPGTSVKVSCKPSGYAFTNYLIDWVKQRPGQGLEWIGGINPGSGDTVYNEKFKAKATLTADKSSMTANMQLSSLTSDDSAVYFCARRVRGNSFDSWGQGTLVTVSA

SEQ ID NO: 156 - protein, 10 aa, Artificial
  Clone 18A9 Heavy Chain CDR1
GYAFTNYLID

SEQ ID NO: 157 - protein, 16 aa, Artificial
  Clone 18A9 Heavy Chain CDR2
GINPGSGDTVYNEKFK

SEQ ID NO: 158 - protein, 9 aa, Artificial
  Clone 18A9 Heavy Chain CDR3
RVRGNSFDS

SEQ ID NO: 159 - protein, 25 aa, Artificial
  Clone 18A9 Heavy Chain FR1
QVQLQQSGREVVRPGTSVKVSCKPS

SEQ ID NO: 160 - protein, 14 aa, Artificial
  Clone 18A9 Heavy Chain FR2
WVKQRPGQGLEWIG

SEQ ID NO: 161 - protein, 33 aa, Artificial
  Clone 18A9 Heavy Chain FR3
AKATLTADKSSMTANMQLSSLTSDDSAVYFCAR

SEQ ID NO: 162 - protein, 11 aa, Artificial
  Clone 18A9 Heavy Chain FR4
WGQGTLVTVSA

SEQ ID NO: 163 - protein, 113 aa, Artificial
  Clone 18A9 Light chain
DIVMSQSPSSLTVTAGEKVTMSCKSSQSLLNSGNQKNYLTWYQQKPGQPPKLLIYWASTRESGVPDRFTGSGSGKDFTLTISSVQAEDLALYYCQNNYFYPLTFGAGTKLELK

SEQ ID NO: 164 - protein, 17 aa, Artificial
  Clone 18A9 Light chain CDR1
KSSQSLLNSGNQKNYLT

SEQ ID NO: 165 - protein, 7 aa, Artificial
  Clone 18A9 Light chain CDR2
WASTRES

SEQ ID NO: 166 - protein, 9 aa, Artificial
  Clone 18A9 Light chain CDR3
QNNYFYPLT

SEQ ID NO: 167 - protein, 23 aa, Artificial
  Clone 18A9 Light chain FR1
DIVMSQSPSSLTVTAGEKVTMSC

SEQ ID NO: 168 - protein, 15 aa, Artificial
  Clone 18A9 Light chain FR2
WYQQKPGQPPKLLIY

SEQ ID NO: 169 - protein, 32 aa, Artificial
  Clone 18A9 Light chain FR3
GVPDRFTGSGSGKDFTLTISSVQAEDLALYYC

SEQ ID NO: 170 - protein, 10 aa, Artificial
  Clone 18A9 Light chain FR4
FGAGTKLELK

SEQ ID NO: 171 - DNA, 37 bp, Artificial
  upstream primer
ttggcaaagaattgctagatgtccaccaccacatgcc

SEQ ID NO: 172 - DNA, 38 bp, Artificial
  downstream primer
tgttcgggccctcctcgattacacatagtcgtgcttgg

SEQ ID NO: 173 - DNA, 37 bp, Artificial
  upstream primer
ttggcaaagaattgctagatggccgtgactgcctgtc

SEQ ID NO: 174 - DNA, 38 bp, Artificial; identical to SEQ ID NO: 172
  downstream primer

SEQ ID NO: 175 - DNA, 20 bp, Artificial
  primer KNB14
tgtgcgccaccatggccgtg

SEQ ID NO: 176 - DNA, 20 bp, Artificial
  primer KNB15
tggaaggataagattgtacc

SEQ ID NO: 177 - DNA, 20 bp, Artificial
  primer KNB16
tgggtgccattggcctcctg

SEQ ID NO: 178 - DNA, 354 bp, Artificial
  Clone 18D10 Heavy Chain
gatgtgcagcttcaggagtcgggacctggcctggtgaaaccttctcagtctctgtccctcacctgcactgtcactggctactcaatcaccagtaattatgcctggaactggatccgacagtttccaggaaacaaactagagtggatgggctacataaactacagtgggaacactaactataacccatctctcaaaagtcgaatctctatcactcgagacacatccaagaaccagttcttcctgcagttgaattctgtgactgctgaggacacagccacatattattgtgcaacctcctattatggtaattcctttatttactggggccaagggactctggtcactgtctctgca

SEQ ID NO: 179 - DNA, 339 bp, Artificial
  Clone 18D10 Light chain
gacattgtgatgacacagtctccatcctccctgactgtgacagcaggagagaaggtcactatgagctgcaagtccagtcagagtctgttaaacagtggaaatcaaaagaactacttgacctggtaccagcagaaaccagggcagcctcctaaactgttgatctactgggcatccactagggagtctggggtccctgatcgcttcacaggcagtggatctggaacagatttcactctcaccatcagcagtgtgcaggctgaagacctggcagtttattactgtcagaatgcttatagttttccgtggacgttcggtggaggcaccaagctggaaatcaaa

SEQ ID NO: 180 - DNA, 354 bp, Artificial
  Clone 18A9 Heavy Chain
caggtgcagctgcagcagtctggacgtgaggtggtaaggcctgggacttcagtgaaggtgtcctgcaagccttctggatacgccttcactaattacttgatagactgggtaaaacagaggcctggacagggccttgagtggattggagggattaatcctggaagtggtgacactgtgtacaatgagaagttcaaggccaaggcaacactgactgcagacaaatcctccatgactgccaacatgcagctcagcagcctgacatctgatgactctgcggtctatttctgcgcaagaagggtccgtggtaattcgtttgattcctggggccaagggactctggtcactgtctctgca

SEQ ID NO: 181 - DNA, 339 bp, Artificial
  Clone 18A9 Light chain
gacattgtgatgtcacagtctccatcctccctgactgtgacagcaggagagaaggtcactatgagctgcaagtccagtcagagtctgttaaacagtggaaatcaaaagaactacttgacctggtaccagcagaaaccagggcagcctcctaaattgttgatctactgggcatccactagggaatctggggtccctgatcgcttcacaggcagtggatctggaaaagatttcactctcaccatcagcagtgtgcaggctgaagacctggcactttattactgtcagaataattatttttatccgctcacgttcggtgctgggaccaagctggagctgaaa

SEQ ID NO: 182 - DNA, 354 bp, Artificial
  18D10VHv1
caggttcagctgcaagagtctggacctggcctggtcaagcctagcgagacactgagcctgacctgtaccgtgtccggctacagcatcaccagcaactacgcctggaactggatcagacagcctcctggcaaaggcctcgagtggatcggctacatcaactacagcggcaacaccaactacaaccccagcctgaagtccagagtgaccatcagcagagacaccagcaagaaccagttctccctgaagctgagcagcgtgacagccgccgatacagccgtgtactactgtgccacaagctactacggcaacagcttcatctactggggccagggcacactggtcaccgtttcttct

SEQ ID NO: 183 - DNA, 354 bp, Artificial
  18D10VHv2
caggttcagctgcaagagtctggacctggcctggtcaagcctagcgagacactgagcctgacctgtaccgtgtccggcggcagcatcagcagcaactacgcctggaactggatcagacagcctcctggcaaaggcctcgagtggatgggctacatcaactacagcggcaacaccaactacaaccccagcctgaagtccagaatcaccatcagcagagacaccagcaagaaccagttctccctgaagctgagcagcgtgacagccgccgatacagccgtgtactactgtgccacaagctactacggcaacagcttcatctactggggccagggcacactggtcaccgtttcttct

SEQ ID NO: 184 - DNA, 354 bp, Artificial
  18D10VHv3
caggttcagctgcaagagtctggacctggcctggtcaagcctagcgagacactgagcctgacctgtaccgtgtccggcggcagcatcagcagcaactacgcctggaactggatcagacagcctcctggcaaaggcctcgagtggatcggctacatcaactacagcggcaacaccaactacaaccccagcctgaagtccagagtgaccatcagcagagacaccagcaagaaccagttctccctgaagctgagcagcgtgacagccgccgatacagccgtgtactactgtgccacaagctactacggcaacagcttcatctactggggccagggcacactggtcaccgtttcttct

SEQ ID NO: 185 - DNA, 354 bp, Artificial
  18D10VHv4
caggttcagctgcaagagtctggacctggcctggtcaagcctagcgagacactgagcctgacctgtaccgtgtccggcggcagcatcagcagcaactacgcctggaactggatcagacagcctcctggcaaaggcctcgagtggatcggctacatcaactacagcggctacaccaactacaaccccagcctgaagtccagagtgaccatcagcagagacaccagcaagaaccagttctccctgaagctgagcagcgtgacagccgccgatacagccgtgtactactgtgccacaagctactacggcaacagcttcatctactggggccagggcacactggtcaccgtttcttct

SEQ ID NO: 186 - DNA, 354 bp, Artificial
  18D10VHv5
caggttcagctgcaagagtctggacctggcctggtcaagcctagcgagacactgagcctgacctgtaccgtgtccggcggcagcatcagcagcaactacgcctggaactggatcagacagcctcctggcaaaggcctcgagtggatcggctacatcaactacagcggcaacaccgcctacaaccccagcctgaagtccagagtgaccatcagcagagacaccagcaagaaccagttctccctgaagctgagcagcgtgacagccgccgatacagccgtgtactactgtgccacaagctactacggcaacagcttcatctactggggccagggcacactggtcaccgtttcttct

SEQ ID NO: 187 - DNA, 354 bp, Artificial
  18D10VHv6
caggttcagctgcaagagtctggacctggcctggtcaagcctagcgagacactgagcctgacctgtaccgtgtccggcggcagcatcagcagcaactacgcctggaactggatcagacagcctcctggcaaaggcctcgagtggatcggctacatctactacagcggcaacaccaactacaaccccagcctgaagtccagagtgaccatcagcagagacaccagcaagaaccagttctccctgaagctgagcagcgtgacagccgccgatacagccgtgtactactgtgccacaagctactacggcaacagcttcatctactggggccagggcacactggtcaccgtttcttct

SEQ ID NO: 188 - DNA, 339 bp, Artificial
  18D10VLv1
gacatcgtgatgacacagagccctgatagcctggccgtgtctctgggagagagagccaccatcaactgcaagagcagccagagcctgctgaacagcggcaaccagaagaactacctgacctggtatcagcagaagcccggccagcctcctaagctgctgatctactgggccagcaccagagaaagcggcgtgccagatagattcagcggcagcggctctggaaccgacttcaccctgacaatcagctccctgcaggccgaggatgtggccgtgtactactgtcagaacgcctacagcttcccctggacattcggccagggcaccaaggtggaaatcaag

SEQ ID NO: 189 - DNA, 339 bp, Artificial
  18D10VLv2
gacatcgtgatgacacagagccctgatagcctggccgtgtctctgggagagagagccaccatcaactgcaagagcagccagagcctgctgaacagcggcaaccagaagaactacctggcctggtatcagcagaagcccggccagcctcctaagctgctgatctactgggccagcaccagagaaagcggcgtgccagatagattcagcggcagcggctctggaaccgacttcaccctgacaatcagctccctgcaggccgaggatgtggccgtgtactactgtcagcaggcctacagcttcccctggacattcggccagggcaccaaggtggaaatcaag

SEQ ID NO: 190 - DNA, 1347 bp, Artificial
  Heavy chain nucleic acid sequence
caggttcagctgcaagagtctggacctggcctggtcaagcctagcgagacactgagcctgacctgtaccgtgtccggcggcagcatcagcagcaactacgcctggaactggatcagacagcctcctggcaaaggcctcgagtggatcggctacatctactacagcggcaacaccaactacaaccccagcctgaagtccagagtgaccatcagcagagacaccagcaagaaccagttctccctgaagctgagcagcgtgacagccgccgatacagccgtgtactactgtgccacaagctactacggcaacagcttcatctactggggccagggcacactggtcaccgtttcttctgctagcaccaagggcccatccgtcttccccctggcaccctcctccaagagcacctctgggggcacagcggccctgggctgcctggtcaaggactacttccccgaaccggtgacggtgtcgtggaactcaggcgccctgaccagcggcgtgcacaccttcccggctgtcctacagtcctcaggactctactccctcagcagcgtggtgaccgtgccctccagcagcttgggcacccagacctacatctgcaacgtgaatcacaagcccagcaacaccaaggtggacaagagagttgagcccaaatcttgtgacaaaactcacacatgcccaccgtgcccagcacctgaactcctggggggaccgtcagtcttcctcttccccccaaaacccaaggacaccctcatgatctcccggacccctgaggtcacatgcgtggtggtggacgtgagccacgaagaccctgaggtcaagttcaactggtacgtggacggcgtggaggtgcataatgccaagacaaagccgcgggaggagcagtacaacagcacgtaccgtgtggtcagcgtcctcaccgtcctgcaccaggactggctgaatggcaaggagtacaagtgcaaggtctccaacaaagccctcccagcccccatcgagaaaaccatctccaaagccaaagggcagccccgagaaccacaggtgtacaccctgcccccatcccgggaggagatgaccaagaaccaggtcagcctgacctgcctggtcaaaggcttctatcccagcgacatcgccgtggagtgggagagcaatgggcagccggagaacaactacaagaccacgcctcccgtgctggactccgacggctccttcttcctctatagcaagctcaccgtggacaagagcaggtggcagcaggggaacgtcttctcatgctccgtgatgcatgaggctctgcacaaccactacacgcagaagtccctctccctgtctccgggtaaatga

SEQ ID NO: 191 - DNA, 663 bp, Artificial
  Light chain nucleic acid sequence
gacatcgtgatgacacagagccctgatagcctggccgtgtctctgggagagagagccaccatcaactgcaagagcagccagagcctgctgaacagcggcaaccagaagaactacctgacctggtatcagcagaagcccggccagcctcctaagctgctgatctactgggccagcaccagagaaagcggcgtgccagatagattcagcggcagcggctctggaaccgacttcaccctgacaatcagctccctgcaggccgaggatgtggccgtgtactactgtcagaacgcctacagcttcccctggacattcggccagggcaccaaggtggaaatcaagcgaactgtggctgcaccatctgtcttcatcttcccgccatctgatgagcagttgaaatctggaactgcctctgttgtgtgcctgctgaataacttctatcccagagaggccaaagtacagtggaaggtggataacgccctccaatcgggtaactcccaggagagtgtcacagagcaggacagcaaggacagcacctacagcctcagcagcaccctgacgctgagcaaagcagactacgagaaacacaaagtctacgcctgcgaagtcacccatcagggcctgagctcgcccgtcacaaagagcttcaacaggggagagtgttag

SEQ ID NO: 192 - DNA, 354 bp, Artificial
  18A9VHv1
caggttcagctggttcagtctggcgccgaagtgaagaaacctggcagcagcgtgaaggtgtcctgcaagccttctggctacgccttcaccaactacctgatcgactgggtccgacaggctcctggacagggacttgaatggatgggcggcatcaaccctggcagcggcgatacagtgtacaacgagaagttccagggcagagtgaccctgaccgccgacaagtctagcatgaccgcctacatggaactgagcagcctgagaagcgaggataccgccgtgtacttctgtgccagaagagtgcggggcaacagcttcgattcttggggccagggaaccctggtcaccgtttcttct

SEQ ID NO: 193 - DNA, 354 bp, Artificial
  18A9VHv2
caggttcagctggttcagtctggcgccgaagtgaagaaacctggcagcagcgtgaaggtgtcctgcaagccttctggctacaccttcaccaactacctgatcgactgggtccgacaggctcctggacagggacttgaatggatgggcggcatcaaccctggcagcggcgatacagtgtacaacgagaagttccagggcagagtgaccctgaccgccgacgagtctaccagcaccgcctacatggaactgagcagcctgagaagcgaggataccgccgtgtacttctgtgccagaagagtgcggggcaacagcttcgattcttggggccagggaaccctggtcaccgtttcttct

SEQ ID NO: 194 - DNA, 354 bp, Artificial
  18A9VHv3
caggttcagctggttcagtctggcgccgaagtgaagaaacctggcagcagcgtgaaggtgtcctgcaagccttctggctacaccttcaccaactacctgatcgactgggtccgacaggctcctggacagggacttgaatggatgggcggcatcaaccctggcagcggcgatacagtgtacaacgagaagttccagggcagagtgaccctgaccgccgacaagtctagcatgaccgcctacatggaactgagcagcctgagaagcgaggataccgccgtgtactactgtgccagaagagtgcggggcaacagcttcgattcttggggccagggaaccctggtcaccgtttcttct

SEQ ID NO: 195 - DNA, 354 bp, Artificial
  18A9VHv4
caggttcagctggttcagtctggcgccgaagtgaagaaacctggcagcagcgtgaaggtgtcctgcaaggcttctggctacaccttcaccaactacctgatcgactgggtccgacaggctcctggacagggacttgaatggatgggcggcatcaaccctggcagcggcgatacagtgtacaacgagaagttccagggcagagtgaccctgaccgccgacaagtctagcatgaccgcctacatggaactgagcagcctgagaagcgaggataccgccgtgtacttctgtgccagaagagtgcggggcaacagcttcgattcttggggccagggaaccctggtcaccgtttcttct

SEQ ID NO: 196 - DNA, 354 bp, Artificial
  18A9VHv5
caggttcagctggttcagtctggcgccgaagtgaagaaacctggcagcagcgtgaaggtgtcctgcaagccttctggctacaccttcaccaactacctgatcgactgggtccgacaggctcctggacagggacttgaatggatgggcggcatcaaccctggcagcggcgatacagtgtacaacgagaagttccagggcagagtgaccatcaccgccgacgagtctaccagcaccgcctacatggaactgagcagcctgagaagcgaggataccgccgtgtacttctgtgccagaagagtgcggggcaacagcttcgattcttggggccagggaaccctggtcaccgtttcttct

SEQ ID NO: 197 - DNA, 354 bp, Artificial
  18A9VHv6
caggttcagctggttcagtctggcgccgaagtgaagaaacctggcgccagcgtgaaggtgtcctgcaagccttctggctacgccttcaccaactacctgatcgactgggtccgacaggctcctggacagggacttgaatggatgggcggcatcaaccctggcagcggcgatacagtgtacaacgagaagttccagggcagagtgaccctgaccgccgacaagtctagcagcaccgcctacatggaactgagcagcctgagaagcgaggataccgccgtgtacttctgtgccagaagagtgcggggcaacagcttcgattcttggggccagggaaccctggtcaccgtttcttct

SEQ ID NO: 198 - DNA, 354 bp, Artificial
  18A9VHv7
caggttcagctggttcagtctggcgccgaagtgaagaaacctggcgccagcgtgaaggtgtcctgcaagccttctggctacaccttcaccaactacctgatcgactgggtccgacaggctcctggacagggacttgaatggatgggcggcatcaaccctggcagcggcgatacagtgtacaacgagaagttccagggcagagtgaccctgaccgccgacacctctaccagcaccgtctacatggaactgagcagcctgagaagcgaggataccgccgtgtacttctgtgccagaagagtgcggggcaacagcttcgattcttggggccagggaaccctggtcaccgtttcttct

SEQ ID NO: 199 - DNA, 339 bp, Artificial
  18A9VLv1
gacatcgtgatgacacagagccctgatagcctggccgtgtctctgggagagagagccaccatcaactgcaagagcagccagagcctgctgaacagcggcaaccagaagaactacctgacctggtatcagcagaagcccggccagcctcctaagctgctgatctactgggccagcaccagagaaagcggcgtgccagatagattcagcggcagcggctctggaaaggacttcaccctgacaatcagctccctgcaggccgaggatgtggccgtgtactactgccagaacaactacttctaccctctgaccttcggcggaggcaccaaggtggaaatcaag

SEQ ID NO: 200 - DNA, 339 bp, Artificial
  18A9VLv2
gacatcgtgatgacacagagccctgatagcctggccgtgtctctgggagagagagccaccatcaactgcaagagcagccagagcctgctgaacagcggcaaccagaagaactacctggcctggtatcagcagaagcccggccagcctcctaagctgctgatctactgggccagcaccagagaaagcggcgtgccagatagattcagcggcagcggctctggaaccgacttcaccctgacaatcagctccctgcaggccgaggatgtggccgtgtactactgccagcagaactacttctaccctctgaccttcggcggaggcaccaaggtggaaatcaag